European Patent Specification EP 3 271 384 B1, published July 26, 2023. Title: Genic sequence encoding a TCR specific for the human MHC class I complex  specific for the HLA-A02 complex and the peptide hTERT865-873, and its use in the engineering of T lymphocyte s for possibile clinical applications of adoptive transfer. Applicant: Università degli Studi di Verona. The sequence listing filed with the application follows.

SEQUENCE LISTING (7 sequences)

SEQ ID NO: 1 - DNA, 816 bp, Artificial Sequence
  TCR catena alpha5 - TCR anti telomerasi epitopo hTERT865-873 ristretto per aplotipo : A2-02*01
atgaagacagtgactggacctttgttcctgtgcttctggctgcagctgaactgtgtgagcagaggcgagcaggtggagcagcgccctcctcacctgagtgtccgggagggagacagtgccgttatcatctgcacctacacagaccctaacagttattacttcttctggtacaagcaagagccgggggcaggtcttcagttgcttatgaaggttttctcaagtacggaaataaacgaaggacaaggattcactgtcctactgaacaagaaagacaaacaactctctctgaacctcacagctgcccatcctggggactcagccgtgtacttctgcgcagtcaggcatgactcgggatacaacaaactcacttttggaaagggcacggtgcttctagtctctccagacatccagaacccagaacctgctgtgtaccagttaaaagatcctcggtctcaggacagcaccctctgcctgttcaccgactttgactcccaaatcaatgtgccgaaaaccatggaatctggaacgttcatcactgacaaaactgtgctggacatgaaagctatggattccaagagcaatggggccattgcctggagcaaccagacaagcttcacctgccaagatatcttcaaagagaccaacgccacctaccccagttcagacgttccctgtgatgccacgttgactgagaaaagctttgaaacagatatgaacctaaactttcaaaacctgtcagttatgggactccgaatcctcctgctgaaagtagccggatttaacctgctcatgacgctgaggctgtggtccagttga

SEQ ID NO: 2 - DNA, 924 bp, Artificial Sequence
  TCR catena beta3 - TCR anti telomerasi epitopo hTERT865-873 ristretto per aplotipo : A2-02*01
atggctacaaggctcctctgttacacagtactttgtctcctgggtgcaagaattttgaattcaaaagtcattcagactccaagatatctggtgaaagggcaaggacaaaaagcaaagatgaggtgtatccctgaaaagggacatccagttgtattctggtatcaacaaaataagaacaatgagtttaaatttttgattaactttcagaatcaagaagttcttcagcaaatagacatgactgaaaaacgattctctgctgagtgtccttcaaactcaccttgcagcctagaaattcagtcctctgaggcaggagactcagcactgtacctctgtgccagcagtctgtcgaagggggggttctatgaacagtacttcggtcccggcaccaggctcacggttttagaggatctgagaaatgtgactccacccaaggtctccttgtttgagccatcaaaagcagagattgcaaacaaacaaaaggctaccctcgtgtgcttggccaggggcttcttccctgaccacgtggagctgagctggtgggtgaatggcaaggaggtccacagtggggtcagcacggaccctcaggcctacaaggagagcaattatagctactgcctgagcagccgcctgagggtctctgctaccttctggcacaatcctcgaaaccacttccgctgccaagtgcagttccatgggctttcagaggaggacaagtggccagagggctcacccaaacctgtcacacagaacatcagtgcagaggcctggggccgagcagactgtggaatcacttcagcatcctatcatcagggggttctgtctgcaaccatcctctatgagatcctactggggaaggccaccctatatgctgtgctggtcagtggcctggtgctgatggccatggtcaagaaaaaaaattcctga

SEQ ID NO: 3 - DNA, 20 bp, Artificial Sequence
  forward primer
ctaaggccaaccgtgaaaag

SEQ ID NO: 4 - DNA, 20 bp, Artificial Sequence
  reverse primer
ggagagcatagccctcgtag

SEQ ID NO: 5 - DNA, 23 bp, Artificial Sequence
  forward primer
ttttcggaattctaagccaccat

SEQ ID NO: 6 - DNA, 25 bp, Artificial Sequence
  reverse primer
gcttaaacgtttgtctcaggaattt

SEQ ID NO: 7 - protein, 9 aa, Homo sapiens
RLVDDFLLV